European Patent Application EP 4 335 921 A1, published March 13, 2024. Title: WASCH- UND REINIGUNGSMITTEL ENTHALTEND TANNASE II. Applicant: Henkel AG & KGaA. The sequence listing filed with the application follows.

SEQUENCE LISTING (1 sequence)

SEQ ID NO: 1 - protein, 679 aa, Paenibacillus pabuli
MKTKKWVASLLALALMSMPLVSVASAATSTENKLYSLDFDTTNYTEKSLTYNGQTIKYRAYEKIVYVQRPVDTQYEIMNIYVPEEYFEGGTINNYTADTAPIYFPNTVAGYLPGTPGSPGQGMGGGENAIVALSKGYVVAEPGARGRTTQDEDGTYTGKAPAAIVDLKAAVRYLRYNDEVMPGDAEKIISDGTSAGGAMSALLGATGNDADYEPYLEELGAADERDDIYASAVYTPITDLEHADMAYEWQFNGVNTVTPRTFGLAAGQGGPKTSEDGLPELSEGDSPELPEGGLPEGGMPGGMGGNSTPTKLTEDEIKVSDDLSAMFPSYLNSLGLTAPDGTALTLGSDGNGTFKEYVKSYVIASAQKALDEGIDLSDKTWITIENGTVSDIDFDQYITYLTRMKSPSAFDGLDLGNGENQLFGTDTIDNQHFTEYGMENDTAGGTMADSELIKIMNPLNYIDTEGADTSTYWRIRFGTKDSDTSLAVSTILATTLQNKGYNVDFAMPWDVTHSGDYDLEELFAWADQIVAKSSSESDDDQSKTSDNITVKVNNEDVAASTYEHDGSVYLKLRDLAMAVTGSDKQFEITWEPTKKTVNLVSGKSYTPNGGELAGTTSLASEQVTSKASTIYLDGQQVQLTAYMVQGNNYVKLSEAANLLNLDLVIDSTTNTVTINTVEN